European Patent Specification EP 3 603 622 B1, published March 8, 2023. Title: BIOMATRIX SCAFFOLDS FOR INDUSTRIAL SCALE DISPERSAL. Applicant: University of North Carolina at Chapel Hill Roach, Marsha Lynn Malavarca, Richard Harold. The sequence listing filed with the application follows.

SEQUENCE LISTING (34 sequences)

SEQ ID NO: 1 - DNA, 21 bp, Artificial Sequence
  RT-PCR primer
tacaccgaggaaatgggctca

SEQ ID NO: 2 - DNA, 22 bp, Artificial Sequence
  RT-PCR primer
agatgatggagtagatggtggg

SEQ ID NO: 3 - DNA, 21 bp, Artificial Sequence
  RT-PCR primer
ataacctgctctgagcgagtg

SEQ ID NO: 4 - DNA, 20 bp, Artificial Sequence
  RT-PCR primer
tgaagtgcagtccgcaaact

SEQ ID NO: 5 - DNA, 21 bp, Artificial Sequence
  RT-PCR primer
accaagtttgagacggaacag

SEQ ID NO: 6 - DNA, 21 bp, Artificial Sequence
  RT-PCR primer
ccctcagcgtactgatttcct

SEQ ID NO: 7 - DNA, 20 bp, Artificial Sequence
  RT-PCR primer
atgtggaagtggctgcagga

SEQ ID NO: 8 - DNA, 21 bp, Artificial Sequence
  RT-PCR primer
tgtgttgcctctatccttccc

SEQ ID NO: 9 - DNA, 19 bp, Artificial Sequence
  RT-PCR primer
gcgaccccaagacctacag

SEQ ID NO: 10 - DNA, 19 bp, Artificial Sequence
  RT-PCR primer
ggttctgccggtagaaggg

SEQ ID NO: 11 - DNA, 23 bp, Artificial Sequence
  RT-PCR primer
ttgacattggagtgaaaaggacg

SEQ ID NO: 12 - DNA, 21 bp, Artificial Sequence
  RT-PCR primer
tgctcagaaccttggggattc

SEQ ID NO: 13 - DNA, 21 bp, Artificial Sequence
  RT-PCR primer
cttgcacacaaaaagcccact

SEQ ID NO: 14 - DNA, 23 bp, Artificial Sequence
  RT-PCR primer
gggatgccttcttgctatctcat

SEQ ID NO: 15 - DNA, 21 bp, Artificial Sequence
  RT-PCR primer
tttatgccccggaactccttt

SEQ ID NO: 16 - DNA, 21 bp, Artificial Sequence
  RT-PCR primer
acaggcaggcagctttatcag

SEQ ID NO: 17 - DNA, 22 bp, Artificial Sequence
  RT-PCR primer
cctcctaccttgattgcatcag

SEQ ID NO: 18 - DNA, 22 bp, Artificial Sequence
  RT-PCR primer
ttttgacccatagaactctgcc

SEQ ID NO: 19 - DNA, 21 bp, Artificial Sequence
  RT-PCR primer
aagtcgcctcgaagatacaca

SEQ ID NO: 20 - DNA, 21 bp, Artificial Sequence
  RT-PCR primer
aaggagagaacactgctcgtg

SEQ ID NO: 21 - DNA, 21 bp, Artificial Sequence
  RT-PCR primer
tttgggaccctgtaccattgt

SEQ ID NO: 22 - DNA, 21 bp, Artificial Sequence
  RT-PCR primer
gcattggacttgaggaagctc

SEQ ID NO: 23 - DNA, 22 bp, Artificial Sequence
  RT-PCR primer
tcagggaaagataaagccgacc

SEQ ID NO: 24 - DNA, 23 bp, Artificial Sequence
  RT-PCR primer
aggtagattcgtgacagacagac

SEQ ID NO: 25 - DNA, 20 bp, Artificial Sequence
  RT-PCR primer
aaaaggccagcgttgtctcc

SEQ ID NO: 26 - DNA, 21 bp, Artificial Sequence
  RT-PCR primer
tgaagccagctctctatccca

SEQ ID NO: 27 - DNA, 21 bp, Artificial Sequence
  RT-PCR primer
ggggagatcgagggctatgag

SEQ ID NO: 28 - DNA, 21 bp, Artificial Sequence
  RT-PCR primer
gatgacggtccgcttgttttc

SEQ ID NO: 29 - DNA, 19 bp, Artificial Sequence
  RT-PCR primer
gccaagggcgcagattctt

SEQ ID NO: 30 - DNA, 19 bp, Artificial Sequence
  RT-PCR primer
ccagggtgcggtgaagttc

SEQ ID NO: 31 - DNA, 21 bp, Artificial Sequence
  RT-PCR primer
tgtgttggcttcctctgtcag

SEQ ID NO: 32 - DNA, 22 bp, Artificial Sequence
  RT-PCR primer
ggcagcatcctataatgagcac

SEQ ID NO: 33 - DNA, 23 bp, Artificial Sequence
  RT-PCR primer
catgagaagtatgacaacagcct

SEQ ID NO: 34 - DNA, 22 bp, Artificial Sequence
  RT-PCR primer
agtccttccacgataccaaagt